European Patent Application EP 4 273 227 A1, published November 8, 2023. Title: Recombinant strain with Modified Gene BBD29_04920 for Producing L-Glutamic Acid, and Method for Constructing the Same and Use Thereof. Applicant: INNER MONGOLIA EPPEN BIOTECH CO., LTD. The sequence listing filed with the application follows.

SEQUENCE LISTING (46 sequences)

SEQ ID NO: 1 - DNA, 1788 bp, Corynebacterium glutamicum
atgactacatctgacccaaattcgaaaccgatagtggaggatgctcagccagagcagatcaccgcaaccgaagaactggcgggtttgcttgagaatccaactaacctggaagggaaactggccgacgccgaagaggaaattatcctcgaaggcgaagacgcccaggcctcacttaactggtcagtcatcgttccagccctagtcattgtcctagcgacagtggtgtggggtatcggattcaaagatagctttaccaactttgctagttctgcgttgtcagcagtagttgacaatctcggctgggccttcattttgtttggcacagtctttgtattttttatcgttgttatcgccgctagtaaattcggcacgattcgcttaggccgcattgatgaagcaccagagtttcgcacggtgtcatggatttccatgatgtttgctgcaggtatgggtattggtttgatgttctacggaaccacagaacctttaaccttctaccgcaatggtgtacctggatatgatgaacacaatgttggcgttgctatgtccacgacaatgttccactggaccttgcatccatgggctatctacgcaattgtgggcctagccattgcctattcgaccttccgagtgggccgtaaacagcttctaagctctgcattcgtgccactcattggtgaaaaaggtgcagaaggatggttgggcaagctcatcgacatcctggcgattatcgccacagtattcggcaccgcatgttcccttggcctgggtgcgctgcagatcggtgcaggactttccgcagccaacatcattgaaaatccgagtgactggactgtcattggtattgtttctgtcttgaccttggcatttatcttctctgctatttctggtgtgggcaagggaatccagtacctctccaacgccaacatggttctggcagctctgctcgcgattttcgtgttcgttgtcggaccaaccgtgtcgattttgaacctgctgccaggttctattggcaactacctgtccaacttcttccaaatggcaggccgcactgccatgagtgccgacggcacagcaggtgagtggctaggtagctggaccatcttctactgggcatggtggatctcttggtcaccattcgtaggaatgttcttggcacgtatttcccgtggccgctccatccgtgagttcatcctgggcgtgttgctcgtcccagcaggtgtgtccaccgtatggttctccatttttggtggcactgcgattgtcttcgaacaaaatggggaatccatttggggtgatggtgcagcagaagagcagctctttggattgcttcatgcacttccaggtgggcaaataatgggcatcatcgccatgattttgctgggtactttcttcattacctctgcagactctgcttccaccgtcatgggcaccatgagtcagcacggccagctggaagccaacaagtgggtgacagctgcctggggtgttgctaccgcagctattggactaacgctattgctttctggtggtgacaatgccttgaacaacttgcaaaacgtcaccatcgtggctgcaacaccattcctgtttgtggttattggattgatgtttgcgttagtcaaggacttaagcaatgatgtgatctacctcgagtaccgtgagcagcaacgcttcaacgcgcgccttgcccgtgaacgtcgtgttcacaatgaacaccgcaagcgtgaactggctgcaaagcgacgcagggagcgtaaggcgagtggcgcggggaagcgtcgatag

SEQ ID NO: 2 - DNA, 1788 bp, Artificial Sequence
  BBD29_04920C1560A ORF sequence
atgactacatctgacccaaattcgaaaccgatagtggaggatgctcagccagagcagatcaccgcaaccgaagaactggcgggtttgcttgagaatccaactaacctggaagggaaactggccgacgccgaagaggaaattatcctcgaaggcgaagacgcccaggcctcacttaactggtcagtcatcgttccagccctagtcattgtcctagcgacagtggtgtggggtatcggattcaaagatagctttaccaactttgctagttctgcgttgtcagcagtagttgacaatctcggctgggccttcattttgtttggcacagtctttgtattttttatcgttgttatcgccgctagtaaattcggcacgattcgcttaggccgcattgatgaagcaccagagtttcgcacggtgtcatggatttccatgatgtttgctgcaggtatgggtattggtttgatgttctacggaaccacagaacctttaaccttctaccgcaatggtgtacctggatatgatgaacacaatgttggcgttgctatgtccacgacaatgttccactggaccttgcatccatgggctatctacgcaattgtgggcctagccattgcctattcgaccttccgagtgggccgtaaacagcttctaagctctgcattcgtgccactcattggtgaaaaaggtgcagaaggatggttgggcaagctcatcgacatcctggcgattatcgccacagtattcggcaccgcatgttcccttggcctgggtgcgctgcagatcggtgcaggactttccgcagccaacatcattgaaaatccgagtgactggactgtcattggtattgtttctgtcttgaccttggcatttatcttctctgctatttctggtgtgggcaagggaatccagtacctctccaacgccaacatggttctggcagctctgctcgcgattttcgtgttcgttgtcggaccaaccgtgtcgattttgaacctgctgccaggttctattggcaactacctgtccaacttcttccaaatggcaggccgcactgccatgagtgccgacggcacagcaggtgagtggctaggtagctggaccatcttctactgggcatggtggatctcttggtcaccattcgtaggaatgttcttggcacgtatttcccgtggccgctccatccgtgagttcatcctgggcgtgttgctcgtcccagcaggtgtgtccaccgtatggttctccatttttggtggcactgcgattgtcttcgaacaaaatggggaatccatttggggtgatggtgcagcagaagagcagctctttggattgcttcatgcacttccaggtgggcaaataatgggcatcatcgccatgattttgctgggtactttcttcattacctctgcagactctgcttccaccgtcatgggcaccatgagtcagcacggccagctggaagccaacaagtgggtgacagctgcctggggtgttgctaccgcagctattggactaacgctattgctttctggtggtgacaatgccttgaacaacttgcaaaaagtcaccatcgtggctgcaacaccattcctgtttgtggttattggattgatgtttgcgttagtcaaggacttaagcaatgatgtgatctacctcgagtaccgtgagcagcaacgcttcaacgcgcgccttgcccgtgaacgtcgtgttcacaatgaacaccgcaagcgtgaactggctgcaaagcgacgcagggagcgtaaggcgagtggcgcggggaagcgtcgatag

SEQ ID NO: 3 - protein, 595 aa, Corynebacterium glutamicum
MTTSDPNSKPIVEDAQPEQITATEELAGLLENPTNLEGKLADAEEEIILEGEDAQASLNWSVIVPALVIVLATVVWGIGFKDSFTNFASSALSAVVDNLGWAFILFGTVFVFFIVVIAASKFGTIRLGRIDEAPEFRTVSWISMMFAAGMGIGLMFYGTTEPLTFYRNGVPGYDEHNVGVAMSTTMFHWTLHPWAIYAIVGLAIAYSTFRVGRKQLLSSAFVPLIGEKGAEGWLGKLIDILAIIATVFGTACSLGLGALQIGAGLSAANIIENPSDWTVIGIVSVLTLAFIFSAISGVGKGIQYLSNANMVLAALLAIFVFVVGPTVSILNLLPGSIGNYLSNFFQMAGRTAMSADGTAGEWLGSWTIFYWAWWISWSPFVGMFLARISRGRSIREFILGVLLVPAGVSTVWFSIFGGTAIVFEQNGESIWGDGAAEEQLFGLLHALPGGQIMGIIAMILLGTFFITSADSASTVMGTMSQHGQLEANKWVTAAWGVATAAIGLTLLLSGGDNALNNLQNVTIVAATPFLFVVIGLMFALVKDLSNDVIYLEYREQQRFNARLARERRVHNEHRKRELAAKRRRERKASGAGKRR

SEQ ID NO: 4 - protein, 595 aa, Artificial Sequence
  mutant protein BBD29_04920C1560A
MTTSDPNSKPIVEDAQPEQITATEELAGLLENPTNLEGKLADAEEEIILEGEDAQASLNWSVIVPALVIVLATVVWGIGFKDSFTNFASSALSAVVDNLGWAFILFGTVFVFFIVVIAASKFGTIRLGRIDEAPEFRTVSWISMMFAAGMGIGLMFYGTTEPLTFYRNGVPGYDEHNVGVAMSTTMFHWTLHPWAIYAIVGLAIAYSTFRVGRKQLLSSAFVPLIGEKGAEGWLGKLIDILAIIATVFGTACSLGLGALQIGAGLSAANIIENPSDWTVIGIVSVLTLAFIFSAISGVGKGIQYLSNANMVLAALLAIFVFVVGPTVSILNLLPGSIGNYLSNFFQMAGRTAMSADGTAGEWLGSWTIFYWAWWISWSPFVGMFLARISRGRSIREFILGVLLVPAGVSTVWFSIFGGTAIVFEQNGESIWGDGAAEEQLFGLLHALPGGQIMGIIAMILLGTFFITSADSASTVMGTMSQHGQLEANKWVTAAWGVATAAIGLTLLLSGGDNALNNLQKVTIVAATPFLFVVIGLMFALVKDLSNDVIYLEYREQQRFNARLARERRVHNEHRKRELAAKRRRERKASGAGKRR

SEQ ID NO: 5 - DNA, 56 bp, Artificial Sequence
  Primer P1
cagtgccaagcttgcatgcctgcaggtcgactctagtgtttctgtcttgaccttgg

SEQ ID NO: 6 - DNA, 30 bp, Artificial Sequence
  Primer P2
agccacgatggtgactttttgcaagttgtt

SEQ ID NO: 7 - DNA, 30 bp, Artificial Sequence
  Primer P3
aacaacttgcaaaaagtcaccatcgtggct

SEQ ID NO: 8 - DNA, 56 bp, Artificial Sequence
  Primer P4
cagctatgaccatgattacgaattcgagctcggtacccacagattgggcaggtgcc

SEQ ID NO: 9 - DNA, 19 bp, Artificial Sequence
  Primer P5
ctattgctttctggtggtg

SEQ ID NO: 10 - DNA, 20 bp, Artificial Sequence
  Primer P6
tcgccttacgctccctgcgt

SEQ ID NO: 11 - DNA, 56 bp, Artificial Sequence
  Primer P7
cagtgccaagcttgcatgcctgcaggtcgactctaggacccgcttgccatacgaag

SEQ ID NO: 12 - DNA, 40 bp, Artificial Sequence
  Primer P8
gcatcacaatgacataacgaatctactcatctgaagaatc

SEQ ID NO: 13 - DNA, 40 bp, Artificial Sequence
  Primer P9
gattcttcagatgagtagattcgttatgtcattgtgatgc

SEQ ID NO: 14 - DNA, 40 bp, Artificial Sequence
  Primer P10
caaaccagagtgcccacgaactatcgacgcttccccgcgc

SEQ ID NO: 15 - DNA, 40 bp, Artificial Sequence
  Primer P11
gcgcggggaagcgtcgatagttcgtgggcactctggtttg

SEQ ID NO: 16 - DNA, 58 bp, Artificial Sequence
  Primer P12
cagctatgaccatgattacgaattcgagctcggtaccccataagaaacaaccacttcc

SEQ ID NO: 17 - DNA, 20 bp, Artificial Sequence
  Primer P13
gtccaaggtgacggccgcac

SEQ ID NO: 18 - DNA, 20 bp, Artificial Sequence
  Primer P14
ctttttcaccaatgagtggc

SEQ ID NO: 19 - DNA, 20 bp, Artificial Sequence
  Primer P15
ccgtaaacagcttctaagct

SEQ ID NO: 20 - DNA, 20 bp, Artificial Sequence
  Primer P16
atattcggcccagcagcagc

SEQ ID NO: 21 - DNA, 56 bp, Artificial Sequence
  Primer P17
gcttgcatgcctgcaggtcgactctagaggatcccctcgttatgtcattgtgatgc

SEQ ID NO: 22 - DNA, 54 bp, Artificial Sequence
  Primer P18
atcaggctgaaaatcttctctcatccgccaaaacctatcgacgcttccccgcgc

SEQ ID NO: 23 - DNA, 55 bp, Artificial Sequence
  Primer P19
cagtgccaagcttgcatgcctgcaggtcgactctagtaaggggcagttggtctcg

SEQ ID NO: 24 - DNA, 40 bp, Artificial Sequence
  Primer P20
gtatcaggggttaaaaattgcttaattttccctggcagaa

SEQ ID NO: 25 - DNA, 40 bp, Artificial Sequence
  Primer P21
ttctgccagggaaaattaagcaatttttaacccctgatac

SEQ ID NO: 26 - DNA, 58 bp, Artificial Sequence
  Primer P22
cagctatgaccatgattacgaattcgagctcggtacccatatcgcgcgacattgcgcg

SEQ ID NO: 27 - DNA, 19 bp, Artificial Sequence
  Primer P23
taaggggcagttggtctcg

SEQ ID NO: 28 - DNA, 20 bp, Artificial Sequence
  Primer P24
atatcgcgcgacattgcgcg

SEQ ID NO: 29 - DNA, 1521 bp, Artificial Sequence
  PCR amplification products
cagtgccaagcttgcatgcctgcaggtcgactctagtgtttctgtcttgaccttggcatttatcttctctgctatttctggtgtgggcaagggaatccagtacctctccaacgccaacatggttctggcagctctgctcgcgattttcgtgttcgttgtcggaccaaccgtgtcgattttgaacctgctgccaggttctattggcaactacctgtccaacttcttccaaatggcaggccgcactgccatgagtgccgacggcacagcaggtgagtggctaggtagctggaccatcttctactgggcatggtggatctcttggtcaccattcgtaggaatgttcttggcacgtatttcccgtggccgctccatccgtgagttcatcctgggcgtgttgctcgtcccagcaggtgtgtccaccgtatggttctccatttttggtggcactgcgattgtcttcgaacaaaatggggaatccatttggggtgatggtgcagcagaagagcagctctttggattgcttcatgcacttccaggtgggcaaataatgggcatcatcgccatgattttgctgggtactttcttcattacctctgcagactctgcttccaccgtcatgggcaccatgagtcagcacggccagctggaagccaacaagtgggtgacagctgcctggggtgttgctaccgcagctattggactaacgctattgctttctggtggtgacaatgccttgaacaacttgcaaaaagtcaccatcgtggctgcaacaccattcctgtttgtggttattggattgatgtttgcgttagtcaaggacttaagcaatgatgtgatctacctcgagtaccgtgagcagcaacgcttcaacgcgcgccttgcccgtgaacgtcgtgttcacaatgaacaccgcaagcgtgaactggctgcaaagcgacgcagggagcgtaaggcgagtggcgcggggaagcgtcgataggcaatttttaacccctgatacccctttccggccgggcataaattaaggtggtacgcatgacgaagaacgtgctcgtatctgttgcctggccgtatgccaacggaccccgtcacattggacatgtggcggggtttggtgtcccctccgatgtgttcgcaaggttccagcgaatgtctggcaacaacgtgctcatggtgtccggcaccgatgagcacggcacgccacttctggttcaagcagacaaagaaggcgtcaccgttcaagacctcgcggataagtacaaccgccagatcgtcgaagacctcaccggcctgggcctgtcctatgaccttttcacccgcaccaccacctccaaccactacgcagtagtgcaggaactgttccgtggtctgtacgacaacggttacatgatcaaggaaaccaccctcggtgcgatttccccatccactggccgtaccctgccagaccgctacattgaaggcacctgcccaatctgtgggtaccgagctcgaattcgtaatcatggtcatagctgtttcctg

SEQ ID NO: 30 - DNA, 250 bp, Artificial Sequence
  PCR amplification products
ctattgctttctggtggtgacaatgccttgaacaacttgcaaaacgtcaccatcgtggctgcaacaccattcctgtttgtggttattggattgatgtttgcgttagtcaaggacttaagcaatgatgtgatctacctcgagtaccgtgagcagcaacgcttcaacgcgcgccttgcccgtgaacgtcgtgttcacaatgaacaccgcaagcgtgaactggctgcaaagcgacgcagggagcgtaaggcga

SEQ ID NO: 31 - DNA, 806 bp, Artificial Sequence
  upstream homologous arm fragment
cagtgccaagcttgcatgcctgcaggtcgactctaggacccgcttgccatacgaagtcctggagaagatctccacccgcatcaccaacgaagttccagacgtaaaccgcgtggttttggacgtaacctccaagccaccaggaaccatcgaatgggagtaggccttaaatgagccttcgttaagcggcaatcaccttatcggtgattgccgctttcccatttctccgggttttctggaactttttgggcgtatgctgggaatgatcttattattttgatttcagaaagcaggagagaccagatgagcgaaatccttgaaacctactgggcaccccacttcggaaacaccgatgaagccgcagcactcgtttcatacttggcacaagcttccggtgatcctattgaggttcacaccctgttcggggatttaggtttagacggactctctggaaactacaccgacactgagatcgacggctacggcgacgcattcctgctggttgcagcactagcagtgttgatggctgaaaacaaagcatccggcggcgtgaatctgggtgaagttgggggagctgataaatcgatccggctgcatgttgaatccaaggaaaacacccagatcaacaccgcattgaagtactttgcgctttccccagaagaccacgcagcggcagatcgcttcgatgaggatgacctgtctgagcttgccaacttgagtgaagagctgcgcggacagctggactaattgctgcccgtttaaggagtccgattcttcagatgagtagattcgttatgtcattgtgatgc

SEQ ID NO: 32 - DNA, 1987 bp, Artificial Sequence
  BBD29_04920 CDS and its promoter fragment
gattcttcagatgagtagattcgttatgtcattgtgatgctcccgtgaacataaacgggacctactggctttacttaagtaacagctatgtaaaagaccaggtcaggttcgggtcggtttaggtacgaaacccatttttcggtttgctttccaggtttccccaagtaaaggtgagttttatgactacatctgacccaaattcgaaaccgatagtggaggatgctcagccagagcagatcaccgcaaccgaagaactggcgggtttgcttgagaatccaactaacctggaagggaaactggccgacgccgaagaggaaattatcctcgaaggcgaagacgcccaggcctcacttaactggtcagtcatcgttccagccctagtcattgtcctagcgacagtggtgtggggtatcggattcaaagatagctttaccaactttgctagttctgcgttgtcagcagtagttgacaatctcggctgggccttcattttgtttggcacagtctttgtattttttatcgttgttatcgccgctagtaaattcggcacgattcgcttaggccgcattgatgaagcaccagagtttcgcacggtgtcatggatttccatgatgtttgctgcaggtatgggtattggtttgatgttctacggaaccacagaacctttaaccttctaccgcaatggtgtacctggatatgatgaacacaatgttggcgttgctatgtccacgacaatgttccactggaccttgcatccatgggctatctacgcaattgtgggcctagccattgcctattcgaccttccgagtgggccgtaaacagcttctaagctctgcattcgtgccactcattggtgaaaaaggtgcagaaggatggttgggcaagctcatcgacatcctggcgattatcgccacagtattcggcaccgcatgttcccttggcctgggtgcgctgcagatcggtgcaggactttccgcagccaacatcattgaaaatccgagtgactggactgtcattggtattgtttctgtcttgaccttggcatttatcttctctgctatttctggtgtgggcaagggaatccagtacctctccaacgccaacatggttctggcagctctgctcgcgattttcgtgttcgttgtcggaccaaccgtgtcgattttgaacctgctgccaggttctattggcaactacctgtccaacttcttccaaatggcaggccgcactgccatgagtgccgacggcacagcaggtgagtggctaggtagctggaccatcttctactgggcatggtggatctcttggtcaccattcgtaggaatgttcttggcacgtatttcccgtggccgctccatccgtgagttcatcctgggcgtgttgctcgtcccagcaggtgtgtccaccgtatggttctccatttttggtggcactgcgattgtcttcgaacaaaatggggaatccatttggggtgatggtgcagcagaagagcagctctttggattgcttcatgcacttccaggtgggcaaataatgggcatcatcgccatgattttgctgggtactttcttcattacctctgcagactctgcttccaccgtcatgggcaccatgagtcagcacggccagctggaagccaacaagtgggtgacagctgcctggggtgttgctaccgcagctattggactaacgctattgctttctggtggtgacaatgccttgaacaacttgcaaaacgtcaccatcgtggctgcaacaccattcctgtttgtggttattggattgatgtttgcgttagtcaaggacttaagcaatgatgtgatctacctcgagtaccgtgagcagcaacgcttcaacgcgcgccttgcccgtgaacgtcgtgttcacaatgaacaccgcaagcgtgaactggctgcaaagcgacgcagggagcgtaaggcgagtggcgcggggaagcgtcgatagttcgtgggcactctggtttg

SEQ ID NO: 33 - DNA, 1987 bp, Artificial Sequence
  BBD29_04920C1560A CDS and its promoter fragment
gattcttcagatgagtagattcgttatgtcattgtgatgctcccgtgaacataaacgggacctactggctttacttaagtaacagctatgtaaaagaccaggtcaggttcgggtcggtttaggtacgaaacccatttttcggtttgctttccaggtttccccaagtaaaggtgagttttatgactacatctgacccaaattcgaaaccgatagtggaggatgctcagccagagcagatcaccgcaaccgaagaactggcgggtttgcttgagaatccaactaacctggaagggaaactggccgacgccgaagaggaaattatcctcgaaggcgaagacgcccaggcctcacttaactggtcagtcatcgttccagccctagtcattgtcctagcgacagtggtgtggggtatcggattcaaagatagctttaccaactttgctagttctgcgttgtcagcagtagttgacaatctcggctgggccttcattttgtttggcacagtctttgtattttttatcgttgttatcgccgctagtaaattcggcacgattcgcttaggccgcattgatgaagcaccagagtttcgcacggtgtcatggatttccatgatgtttgctgcaggtatgggtattggtttgatgttctacggaaccacagaacctttaaccttctaccgcaatggtgtacctggatatgatgaacacaatgttggcgttgctatgtccacgacaatgttccactggaccttgcatccatgggctatctacgcaattgtgggcctagccattgcctattcgaccttccgagtgggccgtaaacagcttctaagctctgcattcgtgccactcattggtgaaaaaggtgcagaaggatggttgggcaagctcatcgacatcctggcgattatcgccacagtattcggcaccgcatgttcccttggcctgggtgcgctgcagatcggtgcaggactttccgcagccaacatcattgaaaatccgagtgactggactgtcattggtattgtttctgtcttgaccttggcatttatcttctctgctatttctggtgtgggcaagggaatccagtacctctccaacgccaacatggttctggcagctctgctcgcgattttcgtgttcgttgtcggaccaaccgtgtcgattttgaacctgctgccaggttctattggcaactacctgtccaacttcttccaaatggcaggccgcactgccatgagtgccgacggcacagcaggtgagtggctaggtagctggaccatcttctactgggcatggtggatctcttggtcaccattcgtaggaatgttcttggcacgtatttcccgtggccgctccatccgtgagttcatcctgggcgtgttgctcgtcccagcaggtgtgtccaccgtatggttctccatttttggtggcactgcgattgtcttcgaacaaaatggggaatccatttggggtgatggtgcagcagaagagcagctctttggattgcttcatgcacttccaggtgggcaaataatgggcatcatcgccatgattttgctgggtactttcttcattacctctgcagactctgcttccaccgtcatgggcaccatgagtcagcacggccagctggaagccaacaagtgggtgacagctgcctggggtgttgctaccgcagctattggactaacgctattgctttctggtggtgacaatgccttgaacaacttgcaaaaagtcaccatcgtggctgcaacaccattcctgtttgtggttattggattgatgtttgcgttagtcaaggacttaagcaatgatgtgatctacctcgagtaccgtgagcagcaacgcttcaacgcgcgccttgcccgtgaacgtcgtgttcacaatgaacaccgcaagcgtgaactggctgcaaagcgacgcagggagcgtaaggcgagtggcgcggggaagcgtcgatagttcgtgggcactctggtttg

SEQ ID NO: 34 - DNA, 788 bp, Artificial Sequence
  Downstream homologous arm fragment
gcgcggggaagcgtcgatagttcgtgggcactctggtttggttaccaggatgggttagtcattctgatcagcgaattccacgttcacatcgccaattccagagttcacaaccagattcagcattggaccttctagatcagcattgtgggcggtgagatctccaacatcacagcgcgctgtgcccacaccggcggtacaacttaggctcacgggcacatcatcgggcagggtgaccatgacttcgccgatccctgaggtgatttggatgttttgttcctgatccaattgggtgaggtggctgaaatcgaggttcatttcacccacgccagaggtgtagctgctgaggagttcatcgttggtggggatgagattgacatcgccgattccagggtcgtcttcaaagtagatgggatcgatatttgaaataaacaggcctgcgagggcgctcatgacaactccggtaccaactacaccgccgacaatccatggccacacatggcgctttttctgaggcttttgtggagggacttgtacatcccaggtgttgtattggttttgggcaagtggatcccaatgaggcgcttcgggggtttgttgcgcgaagggtgcatagtagccctcaacgggggtgatagtgcttagatctggttggggttgtgggtagagatcttcgtttttcatggtggcatcctcagaaacagtgaattcagtggtgagtagtccgcggggtggaagtggttgtttcttatggggtaccgagctcgaattcgtaatcatggtcatagctg

SEQ ID NO: 35 - DNA, 3501 bp, Artificial Sequence
  upstream homologous arm-BBD29_04920-downstream homologous arm
cagtgccaagcttgcatgcctgcaggtcgactctaggacccgcttgccatacgaagtcctggagaagatctccacccgcatcaccaacgaagttccagacgtaaaccgcgtggttttggacgtaacctccaagccaccaggaaccatcgaatgggagtaggccttaaatgagccttcgttaagcggcaatcaccttatcggtgattgccgctttcccatttctccgggttttctggaactttttgggcgtatgctgggaatgatcttattattttgatttcagaaagcaggagagaccagatgagcgaaatccttgaaacctactgggcaccccacttcggaaacaccgatgaagccgcagcactcgtttcatacttggcacaagcttccggtgatcctattgaggttcacaccctgttcggggatttaggtttagacggactctctggaaactacaccgacactgagatcgacggctacggcgacgcattcctgctggttgcagcactagcagtgttgatggctgaaaacaaagcatccggcggcgtgaatctgggtgaagttgggggagctgataaatcgatccggctgcatgttgaatccaaggaaaacacccagatcaacaccgcattgaagtactttgcgctttccccagaagaccacgcagcggcagatcgcttcgatgaggatgacctgtctgagcttgccaacttgagtgaagagctgcgcggacagctggactaattgctgcccgtttaaggagtccgattcttcagatgagtagattcgttatgtcattgtgatgctcccgtgaacataaacgggacctactggctttacttaagtaacagctatgtaaaagaccaggtcaggttcgggtcggtttaggtacgaaacccatttttcggtttgctttccaggtttccccaagtaaaggtgagttttatgactacatctgacccaaattcgaaaccgatagtggaggatgctcagccagagcagatcaccgcaaccgaagaactggcgggtttgcttgagaatccaactaacctggaagggaaactggccgacgccgaagaggaaattatcctcgaaggcgaagacgcccaggcctcacttaactggtcagtcatcgttccagccctagtcattgtcctagcgacagtggtgtggggtatcggattcaaagatagctttaccaactttgctagttctgcgttgtcagcagtagttgacaatctcggctgggccttcattttgtttggcacagtctttgtattttttatcgttgttatcgccgctagtaaattcggcacgattcgcttaggccgcattgatgaagcaccagagtttcgcacggtgtcatggatttccatgatgtttgctgcaggtatgggtattggtttgatgttctacggaaccacagaacctttaaccttctaccgcaatggtgtacctggatatgatgaacacaatgttggcgttgctatgtccacgacaatgttccactggaccttgcatccatgggctatctacgcaattgtgggcctagccattgcctattcgaccttccgagtgggccgtaaacagcttctaagctctgcattcgtgccactcattggtgaaaaaggtgcagaaggatggttgggcaagctcatcgacatcctggcgattatcgccacagtattcggcaccgcatgttcccttggcctgggtgcgctgcagatcggtgcaggactttccgcagccaacatcattgaaaatccgagtgactggactgtcattggtattgtttctgtcttgaccttggcatttatcttctctgctatttctggtgtgggcaagggaatccagtacctctccaacgccaacatggttctggcagctctgctcgcgattttcgtgttcgttgtcggaccaaccgtgtcgattttgaacctgctgccaggttctattggcaactacctgtccaacttcttccaaatggcaggccgcactgccatgagtgccgacggcacagcaggtgagtggctaggtagctggaccatcttctactgggcatggtggatctcttggtcaccattcgtaggaatgttcttggcacgtatttcccgtggccgctccatccgtgagttcatcctgggcgtgttgctcgtcccagcaggtgtgtccaccgtatggttctccatttttggtggcactgcgattgtcttcgaacaaaatggggaatccatttggggtgatggtgcagcagaagagcagctctttggattgcttcatgcacttccaggtgggcaaataatgggcatcatcgccatgattttgctgggtactttcttcattacctctgcagactctgcttccaccgtcatgggcaccatgagtcagcacggccagctggaagccaacaagtgggtgacagctgcctggggtgttgctaccgcagctattggactaacgctattgctttctggtggtgacaatgccttgaacaacttgcaaaacgtcaccatcgtggctgcaacaccattcctgtttgtggttattggattgatgtttgcgttagtcaaggacttaagcaatgatgtgatctacctcgagtaccgtgagcagcaacgcttcaacgcgcgccttgcccgtgaacgtcgtgttcacaatgaacaccgcaagcgtgaactggctgcaaagcgacgcagggagcgtaaggcgagtggcgcggggaagcgtcgatagttcgtgggcactctggtttggttaccaggatgggttagtcattctgatcagcgaattccacgttcacatcgccaattccagagttcacaaccagattcagcattggaccttctagatcagcattgtgggcggtgagatctccaacatcacagcgcgctgtgcccacaccggcggtacaacttaggctcacgggcacatcatcgggcagggtgaccatgacttcgccgatccctgaggtgatttggatgttttgttcctgatccaattgggtgaggtggctgaaatcgaggttcatttcacccacgccagaggtgtagctgctgaggagttcatcgttggtggggatgagattgacatcgccgattccagggtcgtcttcaaagtagatgggatcgatatttgaaataaacaggcctgcgagggcgctcatgacaactccggtaccaactacaccgccgacaatccatggccacacatggcgctttttctgaggcttttgtggagggacttgtacatcccaggtgttgtattggttttgggcaagtggatcccaatgaggcgcttcgggggtttgttgcgcgaagggtgcatagtagccctcaacgggggtgatagtgcttagatctggttggggttgtgggtagagatcttcgtttttcatggtggcatcctcagaaacagtgaattcagtggtgagtagtccgcggggtggaagtggttgtttcttatggggtaccgagctcgaattcgtaatcatggtcatagctg

SEQ ID NO: 36 - DNA, 3501 bp, Artificial Sequence
  upstream homologous arm-BBD29_04920C1560A-downstream homologous arm
cagtgccaagcttgcatgcctgcaggtcgactctaggacccgcttgccatacgaagtcctggagaagatctccacccgcatcaccaacgaagttccagacgtaaaccgcgtggttttggacgtaacctccaagccaccaggaaccatcgaatgggagtaggccttaaatgagccttcgttaagcggcaatcaccttatcggtgattgccgctttcccatttctccgggttttctggaactttttgggcgtatgctgggaatgatcttattattttgatttcagaaagcaggagagaccagatgagcgaaatccttgaaacctactgggcaccccacttcggaaacaccgatgaagccgcagcactcgtttcatacttggcacaagcttccggtgatcctattgaggttcacaccctgttcggggatttaggtttagacggactctctggaaactacaccgacactgagatcgacggctacggcgacgcattcctgctggttgcagcactagcagtgttgatggctgaaaacaaagcatccggcggcgtgaatctgggtgaagttgggggagctgataaatcgatccggctgcatgttgaatccaaggaaaacacccagatcaacaccgcattgaagtactttgcgctttccccagaagaccacgcagcggcagatcgcttcgatgaggatgacctgtctgagcttgccaacttgagtgaagagctgcgcggacagctggactaattgctgcccgtttaaggagtccgattcttcagatgagtagattcgttatgtcattgtgatgctcccgtgaacataaacgggacctactggctttacttaagtaacagctatgtaaaagaccaggtcaggttcgggtcggtttaggtacgaaacccatttttcggtttgctttccaggtttccccaagtaaaggtgagttttatgactacatctgacccaaattcgaaaccgatagtggaggatgctcagccagagcagatcaccgcaaccgaagaactggcgggtttgcttgagaatccaactaacctggaagggaaactggccgacgccgaagaggaaattatcctcgaaggcgaagacgcccaggcctcacttaactggtcagtcatcgttccagccctagtcattgtcctagcgacagtggtgtggggtatcggattcaaagatagctttaccaactttgctagttctgcgttgtcagcagtagttgacaatctcggctgggccttcattttgtttggcacagtctttgtattttttatcgttgttatcgccgctagtaaattcggcacgattcgcttaggccgcattgatgaagcaccagagtttcgcacggtgtcatggatttccatgatgtttgctgcaggtatgggtattggtttgatgttctacggaaccacagaacctttaaccttctaccgcaatggtgtacctggatatgatgaacacaatgttggcgttgctatgtccacgacaatgttccactggaccttgcatccatgggctatctacgcaattgtgggcctagccattgcctattcgaccttccgagtgggccgtaaacagcttctaagctctgcattcgtgccactcattggtgaaaaaggtgcagaaggatggttgggcaagctcatcgacatcctggcgattatcgccacagtattcggcaccgcatgttcccttggcctgggtgcgctgcagatcggtgcaggactttccgcagccaacatcattgaaaatccgagtgactggactgtcattggtattgtttctgtcttgaccttggcatttatcttctctgctatttctggtgtgggcaagggaatccagtacctctccaacgccaacatggttctggcagctctgctcgcgattttcgtgttcgttgtcggaccaaccgtgtcgattttgaacctgctgccaggttctattggcaactacctgtccaacttcttccaaatggcaggccgcactgccatgagtgccgacggcacagcaggtgagtggctaggtagctggaccatcttctactgggcatggtggatctcttggtcaccattcgtaggaatgttcttggcacgtatttcccgtggccgctccatccgtgagttcatcctgggcgtgttgctcgtcccagcaggtgtgtccaccgtatggttctccatttttggtggcactgcgattgtcttcgaacaaaatggggaatccatttggggtgatggtgcagcagaagagcagctctttggattgcttcatgcacttccaggtgggcaaataatgggcatcatcgccatgattttgctgggtactttcttcattacctctgcagactctgcttccaccgtcatgggcaccatgagtcagcacggccagctggaagccaacaagtgggtgacagctgcctggggtgttgctaccgcagctattggactaacgctattgctttctggtggtgacaatgccttgaacaacttgcaaaaagtcaccatcgtggctgcaacaccattcctgtttgtggttattggattgatgtttgcgttagtcaaggacttaagcaatgatgtgatctacctcgagtaccgtgagcagcaacgcttcaacgcgcgccttgcccgtgaacgtcgtgttcacaatgaacaccgcaagcgtgaactggctgcaaagcgacgcagggagcgtaaggcgagtggcgcggggaagcgtcgatagttcgtgggcactctggtttggttaccaggatgggttagtcattctgatcagcgaattccacgttcacatcgccaattccagagttcacaaccagattcagcattggaccttctagatcagcattgtgggcggtgagatctccaacatcacagcgcgctgtgcccacaccggcggtacaacttaggctcacgggcacatcatcgggcagggtgaccatgacttcgccgatccctgaggtgatttggatgttttgttcctgatccaattgggtgaggtggctgaaatcgaggttcatttcacccacgccagaggtgtagctgctgaggagttcatcgttggtggggatgagattgacatcgccgattccagggtcgtcttcaaagtagatgggatcgatatttgaaataaacaggcctgcgagggcgctcatgacaactccggtaccaactacaccgccgacaatccatggccacacatggcgctttttctgaggcttttgtggagggacttgtacatcccaggtgttgtattggttttgggcaagtggatcccaatgaggcgcttcgggggtttgttgcgcgaagggtgcatagtagccctcaacgggggtgatagtgcttagatctggttggggttgtgggtagagatcttcgtttttcatggtggcatcctcagaaacagtgaattcagtggtgagtagtccgcggggtggaagtggttgtttcttatggggtaccgagctcgaattcgtaatcatggtcatagctg

SEQ ID NO: 37 - DNA, 1674 bp, Artificial Sequence
  PCR amplification products
gtccaaggtgacggccgcacctacggacacccaatcgtgctgcgcccagtatcttccgaagacgcaatgaccgccgactggacccgcttgccatacgaagtcctggagaagatctccacccgcatcaccaacgaagttccagacgtaaaccgcgtggttttggacgtaacctccaagccaccaggaaccatcgaatgggagtaggccttaaatgagccttcgttaagcggcaatcaccttatcggtgattgccgctttcccatttctccgggttttctggaactttttgggcgtatgctgggaatgatcttattattttgatttcagaaagcaggagagaccagatgagcgaaatccttgaaacctactgggcaccccacttcggaaacaccgatgaagccgcagcactcgtttcatacttggcacaagcttccggtgatcctattgaggttcacaccctgttcggggatttaggtttagacggactctctggaaactacaccgacactgagatcgacggctacggcgacgcattcctgctggttgcagcactagcagtgttgatggctgaaaacaaagcatccggcggcgtgaatctgggtgaagttgggggagctgataaatcgatccggctgcatgttgaatccaaggaaaacacccagatcaacaccgcattgaagtactttgcgctttccccagaagaccacgcagcggcagatcgcttcgatgaggatgacctgtctgagcttgccaacttgagtgaagagctgcgcggacagctggactaattgctgcccgtttaaggagtccgattcttcagatgagtagattcgttatgtcattgtgatgctcccgtgaacataaacgggacctactggctttacttaagtaacagctatgtaaaagaccaggtcaggttcgggtcggtttaggtacgaaacccatttttcggtttgctttccaggtttccccaagtaaaggtgagttttatgactacatctgacccaaattcgaaaccgatagtggaggatgctcagccagagcagatcaccgcaaccgaagaactggcgggtttgcttgagaatccaactaacctggaagggaaactggccgacgccgaagaggaaattatcctcgaaggcgaagacgcccaggcctcacttaactggtcagtcatcgttccagccctagtcattgtcctagcgacagtggtgtggggtatcggattcaaagatagctttaccaactttgctagttctgcgttgtcagcagtagttgacaatctcggctgggccttcattttgtttggcacagtctttgtattttttatcgttgttatcgccgctagtaaattcggcacgattcgcttaggccgcattgatgaagcaccagagtttcgcacggtgtcatggatttccatgatgtttgctgcaggtatgggtattggtttgatgttctacggaaccacagaacctttaaccttctaccgcaatggtgtacctggatatgatgaacacaatgttggcgttgctatgtccacgacaatgttccactggaccttgcatccatgggctatctacgcaattgtgggcctagccattgcctattcgaccttccgagtgggccgtaaacagcttctaagctctgcattcgtgccactcattggtgaaaaag

SEQ ID NO: 38 - DNA, 1943 bp, Artificial Sequence
  PCR amplification products
ccgtaaacagcttctaagctctgcattcgtgccactcattggtgaaaaaggtgcagaaggatggttgggcaagctcatcgacatcctggcgattatcgccacagtattcggcaccgcatgttcccttggcctgggtgcgctgcagatcggtgcaggactttccgcagccaacatcattgaaaatccgagtgactggactgtcattggtattgtttctgtcttgaccttggcatttatcttctctgctatttctggtgtgggcaagggaatccagtacctctccaacgccaacatggttctggcagctctgctcgcgattttcgtgttcgttgtcggaccaaccgtgtcgattttgaacctgctgccaggttctattggcaactacctgtccaacttcttccaaatggcaggccgcactgccatgagtgccgacggcacagcaggtgagtggctaggtagctggaccatcttctactgggcatggtggatctcttggtcaccattcgtaggaatgttcttggcacgtatttcccgtggccgctccatccgtgagttcatcctgggcgtgttgctcgtcccagcaggtgtgtccaccgtatggttctccatttttggtggcactgcgattgtcttcgaacaaaatggggaatccatttggggtgatggtgcagcagaagagcagctctttggattgcttcatgcacttccaggtgggcaaataatgggcatcatcgccatgattttgctgggtactttcttcattacctctgcagactctgcttccaccgtcatgggcaccatgagtcagcacggccagctggaagccaacaagtgggtgacagctgcctggggtgttgctaccgcagctattggactaacgctattgctttctggtggtgacaatgccttgaacaacttgcaaaacgtcaccatcgtggctgcaacaccattcctgtttgtggttattggattgatgtttgcgttagtcaaggacttaagcaatgatgtgatctacctcgagtaccgtgagcagcaacgcttcaacgcgcgccttgcccgtgaacgtcgtgttcacaatgaacaccgcaagcgtgaactggctgcaaagcgacgcagggagcgtaaggcgagtggcgcggggaagcgtcgatagttcgtgggcactctggtttggttaccaggatgggttagtcattctgatcagcgaattccacgttcacatcgccaattccagagttcacaaccagattcagcattggaccttctagatcagcattgtgggcggtgagatctccaacatcacagcgcgctgtgcccacaccggcggtacaacttaggctcacgggcacatcatcgggcagggtgaccatgacttcgccgatccctgaggtgatttggatgttttgttcctgatccaattgggtgaggtggctgaaatcgaggttcatttcacccacgccagaggtgtagctgctgaggagttcatcgttggtggggatgagattgacatcgccgattccagggtcgtcttcaaagtagatgggatcgatatttgaaataaacaggcctgcgagggcgctcatgacaactccggtaccaactacaccgccgacaatccatggccacacatggcgctttttctgaggcttttgtggagggacttgtacatcccaggtgttgtattggttttgggcaagtggatcccaatgaggcgcttcgggggtttgttgcgcgaagggtgcatagtagccctcaacgggggtgatagtgcttagatctggttggggttgtgggtagagatcttcgtttttcatggtggcatcctcagaaacagtgaattcagtggtgagtagtccgcggggtggaagtggttgtttcttatgcaacgcccaccacatggctaaaaggcaaaggtaagtaatggctgctgctgggccgaatat

SEQ ID NO: 39 - DNA, 2017 bp, Artificial Sequence
  BBD29_04920 gene and its promoter fragment
gcttgcatgcctgcaggtcgactctagaggatcccctcgttatgtcattgtgatgctcccgtgaacataaacgggacctactggctttacttaagtaacagctatgtaaaagaccaggtcaggttcgggtcggtttaggtacgaaacccatttttcggtttgctttccaggtttccccaagtaaaggtgagttttatgactacatctgacccaaattcgaaaccgatagtggaggatgctcagccagagcagatcaccgcaaccgaagaactggcgggtttgcttgagaatccaactaacctggaagggaaactggccgacgccgaagaggaaattatcctcgaaggcgaagacgcccaggcctcacttaactggtcagtcatcgttccagccctagtcattgtcctagcgacagtggtgtggggtatcggattcaaagatagctttaccaactttgctagttctgcgttgtcagcagtagttgacaatctcggctgggccttcattttgtttggcacagtctttgtattttttatcgttgttatcgccgctagtaaattcggcacgattcgcttaggccgcattgatgaagcaccagagtttcgcacggtgtcatggatttccatgatgtttgctgcaggtatgggtattggtttgatgttctacggaaccacagaacctttaaccttctaccgcaatggtgtacctggatatgatgaacacaatgttggcgttgctatgtccacgacaatgttccactggaccttgcatccatgggctatctacgcaattgtgggcctagccattgcctattcgaccttccgagtgggccgtaaacagcttctaagctctgcattcgtgccactcattggtgaaaaaggtgcagaaggatggttgggcaagctcatcgacatcctggcgattatcgccacagtattcggcaccgcatgttcccttggcctgggtgcgctgcagatcggtgcaggactttccgcagccaacatcattgaaaatccgagtgactggactgtcattggtattgtttctgtcttgaccttggcatttatcttctctgctatttctggtgtgggcaagggaatccagtacctctccaacgccaacatggttctggcagctctgctcgcgattttcgtgttcgttgtcggaccaaccgtgtcgattttgaacctgctgccaggttctattggcaactacctgtccaacttcttccaaatggcaggccgcactgccatgagtgccgacggcacagcaggtgagtggctaggtagctggaccatcttctactgggcatggtggatctcttggtcaccattcgtaggaatgttcttggcacgtatttcccgtggccgctccatccgtgagttcatcctgggcgtgttgctcgtcccagcaggtgtgtccaccgtatggttctccatttttggtggcactgcgattgtcttcgaacaaaatggggaatccatttggggtgatggtgcagcagaagagcagctctttggattgcttcatgcacttccaggtgggcaaataatgggcatcatcgccatgattttgctgggtactttcttcattacctctgcagactctgcttccaccgtcatgggcaccatgagtcagcacggccagctggaagccaacaagtgggtgacagctgcctggggtgttgctaccgcagctattggactaacgctattgctttctggtggtgacaatgccttgaacaacttgcaaaacgtcaccatcgtggctgcaacaccattcctgtttgtggttattggattgatgtttgcgttagtcaaggacttaagcaatgatgtgatctacctcgagtaccgtgagcagcaacgcttcaacgcgcgccttgcccgtgaacgtcgtgttcacaatgaacaccgcaagcgtgaactggctgcaaagcgacgcagggagcgtaaggcgagtggcgcggggaagcgtcgataggttttggcggatgagagaagattttcagcctgat

SEQ ID NO: 40 - DNA, 2017 bp, Artificial Sequence
  BBD29_04920C1560A gene and its promoter fragment
gcttgcatgcctgcaggtcgactctagaggatcccctcgttatgtcattgtgatgctcccgtgaacataaacgggacctactggctttacttaagtaacagctatgtaaaagaccaggtcaggttcgggtcggtttaggtacgaaacccatttttcggtttgctttccaggtttccccaagtaaaggtgagttttatgactacatctgacccaaattcgaaaccgatagtggaggatgctcagccagagcagatcaccgcaaccgaagaactggcgggtttgcttgagaatccaactaacctggaagggaaactggccgacgccgaagaggaaattatcctcgaaggcgaagacgcccaggcctcacttaactggtcagtcatcgttccagccctagtcattgtcctagcgacagtggtgtggggtatcggattcaaagatagctttaccaactttgctagttctgcgttgtcagcagtagttgacaatctcggctgggccttcattttgtttggcacagtctttgtattttttatcgttgttatcgccgctagtaaattcggcacgattcgcttaggccgcattgatgaagcaccagagtttcgcacggtgtcatggatttccatgatgtttgctgcaggtatgggtattggtttgatgttctacggaaccacagaacctttaaccttctaccgcaatggtgtacctggatatgatgaacacaatgttggcgttgctatgtccacgacaatgttccactggaccttgcatccatgggctatctacgcaattgtgggcctagccattgcctattcgaccttccgagtgggccgtaaacagcttctaagctctgcattcgtgccactcattggtgaaaaaggtgcagaaggatggttgggcaagctcatcgacatcctggcgattatcgccacagtattcggcaccgcatgttcccttggcctgggtgcgctgcagatcggtgcaggactttccgcagccaacatcattgaaaatccgagtgactggactgtcattggtattgtttctgtcttgaccttggcatttatcttctctgctatttctggtgtgggcaagggaatccagtacctctccaacgccaacatggttctggcagctctgctcgcgattttcgtgttcgttgtcggaccaaccgtgtcgattttgaacctgctgccaggttctattggcaactacctgtccaacttcttccaaatggcaggccgcactgccatgagtgccgacggcacagcaggtgagtggctaggtagctggaccatcttctactgggcatggtggatctcttggtcaccattcgtaggaatgttcttggcacgtatttcccgtggccgctccatccgtgagttcatcctgggcgtgttgctcgtcccagcaggtgtgtccaccgtatggttctccatttttggtggcactgcgattgtcttcgaacaaaatggggaatccatttggggtgatggtgcagcagaagagcagctctttggattgcttcatgcacttccaggtgggcaaataatgggcatcatcgccatgattttgctgggtactttcttcattacctctgcagactctgcttccaccgtcatgggcaccatgagtcagcacggccagctggaagccaacaagtgggtgacagctgcctggggtgttgctaccgcagctattggactaacgctattgctttctggtggtgacaatgccttgaacaacttgcaaaaagtcaccatcgtggctgcaacaccattcctgtttgtggttattggattgatgtttgcgttagtcaaggacttaagcaatgatgtgatctacctcgagtaccgtgagcagcaacgcttcaacgcgcgccttgcccgtgaacgtcgtgttcacaatgaacaccgcaagcgtgaactggctgcaaagcgacgcagggagcgtaaggcgagtggcgcggggaagcgtcgataggttttggcggatgagagaagattttcagcctgat

SEQ ID NO: 41 - DNA, 2056 bp, Artificial Sequence
  PCR amplification products
agcggataacaatttcacacaggaaacagaattaattaagcttgcatgcctgcaggtcgactctagaggatcccctcgttatgtcattgtgatgctcccgtgaacataaacgggacctactggctttacttaagtaacagctatgtaaaagaccaggtcaggttcgggtcggtttaggtacgaaacccatttttcggtttgctttccaggtttccccaagtaaaggtgagttttatgactacatctgacccaaattcgaaaccgatagtggaggatgctcagccagagcagatcaccgcaaccgaagaactggcgggtttgcttgagaatccaactaacctggaagggaaactggccgacgccgaagaggaaattatcctcgaaggcgaagacgcccaggcctcacttaactggtcagtcatcgttccagccctagtcattgtcctagcgacagtggtgtggggtatcggattcaaagatagctttaccaactttgctagttctgcgttgtcagcagtagttgacaatctcggctgggccttcattttgtttggcacagtctttgtattttttatcgttgttatcgccgctagtaaattcggcacgattcgcttaggccgcattgatgaagcaccagagtttcgcacggtgtcatggatttccatgatgtttgctgcaggtatgggtattggtttgatgttctacggaaccacagaacctttaaccttctaccgcaatggtgtacctggatatgatgaacacaatgttggcgttgctatgtccacgacaatgttccactggaccttgcatccatgggctatctacgcaattgtgggcctagccattgcctattcgaccttccgagtgggccgtaaacagcttctaagctctgcattcgtgccactcattggtgaaaaaggtgcagaaggatggttgggcaagctcatcgacatcctggcgattatcgccacagtattcggcaccgcatgttcccttggcctgggtgcgctgcagatcggtgcaggactttccgcagccaacatcattgaaaatccgagtgactggactgtcattggtattgtttctgtcttgaccttggcatttatcttctctgctatttctggtgtgggcaagggaatccagtacctctccaacgccaacatggttctggcagctctgctcgcgattttcgtgttcgttgtcggaccaaccgtgtcgattttgaacctgctgccaggttctattggcaactacctgtccaacttcttccaaatggcaggccgcactgccatgagtgccgacggcacagcaggtgagtggctaggtagctggaccatcttctactgggcatggtggatctcttggtcaccattcgtaggaatgttcttggcacgtatttcccgtggccgctccatccgtgagttcatcctgggcgtgttgctcgtcccagcaggtgtgtccaccgtatggttctccatttttggtggcactgcgattgtcttcgaacaaaatggggaatccatttggggtgatggtgcagcagaagagcagctctttggattgcttcatgcacttccaggtgggcaaataatgggcatcatcgccatgattttgctgggtactttcttcattacctctgcagactctgcttccaccgtcatgggcaccatgagtcagcacggccagctggaagccaacaagtgggtgacagctgcctggggtgttgctaccgcagctattggactaacgctattgctttctggtggtgacaatgccttgaacaacttgcaaaacgtcaccatcgtggctgcaacaccattcctgtttgtggttattggattgatgtttgcgttagtcaaggacttaagcaatgatgtgatctacctcgagtaccgtgagcagcaacgcttcaacgcgcgccttgcccgtgaacgtcgtgttcacaatgaacaccgcaagcgtgaactggctgcaaagcgacgcagggagcgtaaggcgagtggcgcggggaagcgtcgataggttttggcggatgagagaagattttcagcctgat

SEQ ID NO: 42 - DNA, 733 bp, Artificial Sequence
  upstream homologous arm fragment
cagtgccaagcttgcatgcctgcaggtcgactctagtaaggggcagttggtctcgaactttgaccataatgaacaggcgcgcgtcggcaagcttattgaagccgcacgcacgggcacggtgctggtggtcagcgatgccggcatgcctgtggtttctgatccgggttttgcgcttatcgacgccgcccacgaggcgaacattccggtcacctgcttccccgggccgtcagctgtgccaactgcgttggcattgtcgggccttcacgtgggccgcttcgccttcgacggtttcgcgccgcgcaaacaaggtgcgcgcaccacgtggttggagtcgttgaaaaccgaaaagcgcgcggtatgtttcttcgaatctcctcaccgcatcgcagaaaccctggctcacgcagccgaagttttaggtgaacgacgcgcagcagtgtgccgtgaactgtccaaaacctacgaacaggtaaagcgtggaaccttgccagagttggcagaatgggcacaagatggggtgcgtggcgagatcaccgttgtcatcgaaggcgcgggcgatatcgcggtcgatgtcgattcgcttatcgacgccgcccagcagcgcgtcgattccggcgagcggttgaaagcggtgtgcgcagacctcgcgaaaatccatggcgtgagcaaaaatgaactctacgatgcggttatttctgccagggaaaattaagcaatttttaacccctgatac

SEQ ID NO: 43 - DNA, 814 bp, Artificial Sequence
  downstream homologous arm fragment
ttctgccagggaaaattaagcaatttttaacccctgatacccctttccggccgggcataaattaaggtggtacgcatgacgaagaacgtgctcgtatctgttgcctggccgtatgccaacggaccccgtcacattggacatgtggcggggtttggtgtcccctccgatgtgttcgcaaggttccagcgaatgtctggcaacaacgtgctcatggtgtccggcaccgatgagcacggcacgccacttctggttcaagcagacaaagaaggcgtcaccgttcaagacctcgcggataagtacaaccgccagatcgtcgaagacctcaccggcctgggcctgtcctatgaccttttcacccgcaccaccacctccaaccactacgcagtagtgcaggaactgttccgtggtctgtacgacaacggttacatgatcaaggaaaccaccctcggtgcgatttccccatccactggccgtaccctgccagaccgctacattgaaggcacctgcccaatctgtggcaccgacggcgctcgtggcgaccagtgcgacaactgcggaaaccagctcgatccagcggacctgatcaacccggtgtccaagatcaacggcgaaaccccagagttcgttgagaccgaacacttcctgctcgacctgccagcactagctgaagcactaaccgagtggctgaagggacgcgaagactggcgtccaaacgtgttgaagttctcgctcaacctgctggacgatatccgcccacgcgcaatgtcgcgcgatatgggtaccgagctcgaattcgtaatcatggtcatagctg

SEQ ID NO: 44 - DNA, 1507 bp, Artificial Sequence
  Homologous arm fragment
cagtgccaagcttgcatgcctgcaggtcgactctagtaaggggcagttggtctcgaactttgaccataatgaacaggcgcgcgtcggcaagcttattgaagccgcacgcacgggcacggtgctggtggtcagcgatgccggcatgcctgtggtttctgatccgggttttgcgcttatcgacgccgcccacgaggcgaacattccggtcacctgcttccccgggccgtcagctgtgccaactgcgttggcattgtcgggccttcacgtgggccgcttcgccttcgacggtttcgcgccgcgcaaacaaggtgcgcgcaccacgtggttggagtcgttgaaaaccgaaaagcgcgcggtatgtttcttcgaatctcctcaccgcatcgcagaaaccctggctcacgcagccgaagttttaggtgaacgacgcgcagcagtgtgccgtgaactgtccaaaacctacgaacaggtaaagcgtggaaccttgccagagttggcagaatgggcacaagatggggtgcgtggcgagatcaccgttgtcatcgaaggcgcgggcgatatcgcggtcgatgtcgattcgcttatcgacgccgcccagcagcgcgtcgattccggcgagcggttgaaagcggtgtgcgcagacctcgcgaaaatccatggcgtgagcaaaaatgaactctacgatgcggttatttctgccagggaaaattaagcaatttttaacccctgatacccctttccggccgggcataaattaaggtggtacgcatgacgaagaacgtgctcgtatctgttgcctggccgtatgccaacggaccccgtcacattggacatgtggcggggtttggtgtcccctccgatgtgttcgcaaggttccagcgaatgtctggcaacaacgtgctcatggtgtccggcaccgatgagcacggcacgccacttctggttcaagcagacaaagaaggcgtcaccgttcaagacctcgcggataagtacaaccgccagatcgtcgaagacctcaccggcctgggcctgtcctatgaccttttcacccgcaccaccacctccaaccactacgcagtagtgcaggaactgttccgtggtctgtacgacaacggttacatgatcaaggaaaccaccctcggtgcgatttccccatccactggccgtaccctgccagaccgctacattgaaggcacctgcccaatctgtggcaccgacggcgctcgtggcgaccagtgcgacaactgcggaaaccagctcgatccagcggacctgatcaacccggtgtccaagatcaacggcgaaaccccagagttcgttgagaccgaacacttcctgctcgacctgccagcactagctgaagcactaaccgagtggctgaagggacgcgaagactggcgtccaaacgtgttgaagttctcgctcaacctgctggacgatatccgcccacgcgcaatgtcgcgcgatatgggtaccgagctcgaattcgtaatcatggtcatagctg

SEQ ID NO: 45 - DNA, 1433 bp, Artificial Sequence
  PCR amplification products
taaggggcagttggtctcgaactttgaccataatgaacaggcgcgcgtcggcaagcttattgaagccgcacgcacgggcacggtgctggtggtcagcgatgccggcatgcctgtggtttctgatccgggttttgcgcttatcgacgccgcccacgaggcgaacattccggtcacctgcttccccgggccgtcagctgtgccaactgcgttggcattgtcgggccttcacgtgggccgcttcgccttcgacggtttcgcgccgcgcaaacaaggtgcgcgcaccacgtggttggagtcgttgaaaaccgaaaagcgcgcggtatgtttcttcgaatctcctcaccgcatcgcagaaaccctggctcacgcagccgaagttttaggtgaacgacgcgcagcagtgtgccgtgaactgtccaaaacctacgaacaggtaaagcgtggaaccttgccagagttggcagaatgggcacaagatggggtgcgtggcgagatcaccgttgtcatcgaaggcgcgggcgatatcgcggtcgatgtcgattcgcttatcgacgccgcccagcagcgcgtcgattccggcgagcggttgaaagcggtgtgcgcagacctcgcgaaaatccatggcgtgagcaaaaatgaactctacgatgcggttatttctgccagggaaaattaagcaatttttaacccctgatacccctttccggccgggcataaattaaggtggtacgcatgacgaagaacgtgctcgtatctgttgcctggccgtatgccaacggaccccgtcacattggacatgtggcggggtttggtgtcccctccgatgtgttcgcaaggttccagcgaatgtctggcaacaacgtgctcatggtgtccggcaccgatgagcacggcacgccacttctggttcaagcagacaaagaaggcgtcaccgttcaagacctcgcggataagtacaaccgccagatcgtcgaagacctcaccggcctgggcctgtcctatgaccttttcacccgcaccaccacctccaaccactacgcagtagtgcaggaactgttccgtggtctgtacgacaacggttacatgatcaaggaaaccaccctcggtgcgatttccccatccactggccgtaccctgccagaccgctacattgaaggcacctgcccaatctgtggcaccgacggcgctcgtggcgaccagtgcgacaactgcggaaaccagctcgatccagcggacctgatcaacccggtgtccaagatcaacggcgaaaccccagagttcgttgagaccgaacacttcctgctcgacctgccagcactagctgaagcactaaccgagtggctgaagggacgcgaagactggcgtccaaacgtgttgaagttctcgctcaacctgctggacgatatccgcccacgcgcaatgtcgcgcgatat

SEQ ID NO: 46 - DNA, 3380 bp, Artificial Sequence
  PCR amplification products
taaggggcagttggtctcgaactttgaccataatgaacaggcgcgcgtcggcaagcttattgaagccgcacgcacgggcacggtgctggtggtcagcgatgccggcatgcctgtggtttctgatccgggttttgcgcttatcgacgccgcccacgaggcgaacattccggtcacctgcttccccgggccgtcagctgtgccaactgcgttggcattgtcgggccttcacgtgggccgcttcgccttcgacggtttcgcgccgcgcaaacaaggtgcgcgcaccacgtggttggagtcgttgaaaaccgaaaagcgcgcggtatgtttcttcgaatctcctcaccgcatcgcagaaaccctggctcacgcagccgaagttttaggtgaacgacgcgcagcagtgtgccgtgaactgtccaaaacctacgaacaggtaaagcgtggaaccttgccagagttggcagaatgggcacaagatggggtgcgtggcgagatcaccgttgtcatcgaaggcgcgggcgatatcgcggtcgatgtcgattcgcttatcgacgccgcccagcagcgcgtcgattccggcgagcggttgaaagcggtgtgcgcagacctcgcgaaaatccatggcgtgagcaaaaatgaactctacgatgcggttatttctgccagggaaaattaatcgttatgtcattgtgatgctcccgtgaacataaacgggacctactggctttacttaagtaacagctatgtaaaagaccaggtcaggttcgggtcggtttaggtacgaaacccatttttcggtttgctttccaggtttccccaagtaaaggtgagttttatgactacatctgacccaaattcgaaaccgatagtggaggatgctcagccagagcagatcaccgcaaccgaagaactggcgggtttgcttgagaatccaactaacctggaagggaaactggccgacgccgaagaggaaattatcctcgaaggcgaagacgcccaggcctcacttaactggtcagtcatcgttccagccctagtcattgtcctagcgacagtggtgtggggtatcggattcaaagatagctttaccaactttgctagttctgcgttgtcagcagtagttgacaatctcggctgggccttcattttgtttggcacagtctttgtattttttatcgttgttatcgccgctagtaaattcggcacgattcgcttaggccgcattgatgaagcaccagagtttcgcacggtgtcatggatttccatgatgtttgctgcaggtatgggtattggtttgatgttctacggaaccacagaacctttaaccttctaccgcaatggtgtacctggatatgatgaacacaatgttggcgttgctatgtccacgacaatgttccactggaccttgcatccatgggctatctacgcaattgtgggcctagccattgcctattcgaccttccgagtgggccgtaaacagcttctaagctctgcattcgtgccactcattggtgaaaaaggtgcagaaggatggttgggcaagctcatcgacatcctggcgattatcgccacagtattcggcaccgcatgttcccttggcctgggtgcgctgcagatcggtgcaggactttccgcagccaacatcattgaaaatccgagtgactggactgtcattggtattgtttctgtcttgaccttggcatttatcttctctgctatttctggtgtgggcaagggaatccagtacctctccaacgccaacatggttctggcagctctgctcgcgattttcgtgttcgttgtcggaccaaccgtgtcgattttgaacctgctgccaggttctattggcaactacctgtccaacttcttccaaatggcaggccgcactgccatgagtgccgacggcacagcaggtgagtggctaggtagctggaccatcttctactgggcatggtggatctcttggtcaccattcgtaggaatgttcttggcacgtatttcccgtggccgctccatccgtgagttcatcctgggcgtgttgctcgtcccagcaggtgtgtccaccgtatggttctccatttttggtggcactgcgattgtcttcgaacaaaatggggaatccatttggggtgatggtgcagcagaagagcagctctttggattgcttcatgcacttccaggtgggcaaataatgggcatcatcgccatgattttgctgggtactttcttcattacctctgcagactctgcttccaccgtcatgggcaccatgagtcagcacggccagctggaagccaacaagtgggtgacagctgcctggggtgttgctaccgcagctattggactaacgctattgctttctggtggtgacaatgccttgaacaacttgcaaaacgtcaccatcgtggctgcaacaccattcctgtttgtggttattggattgatgtttgcgttagtcaaggacttaagcaatgatgtgatctacctcgagtaccgtgagcagcaacgcttcaacgcgcgccttgcccgtgaacgtcgtgttcacaatgaacaccgcaagcgtgaactggctgcaaagcgacgcagggagcgtaaggcgagtggcgcggggaagcgtcgataggcaatttttaacccctgatacccctttccggccgggcataaattaaggtggtacgcatgacgaagaacgtgctcgtatctgttgcctggccgtatgccaacggaccccgtcacattggacatgtggcggggtttggtgtcccctccgatgtgttcgcaaggttccagcgaatgtctggcaacaacgtgctcatggtgtccggcaccgatgagcacggcacgccacttctggttcaagcagacaaagaaggcgtcaccgttcaagacctcgcggataagtacaaccgccagatcgtcgaagacctcaccggcctgggcctgtcctatgaccttttcacccgcaccaccacctccaaccactacgcagtagtgcaggaactgttccgtggtctgtacgacaacggttacatgatcaaggaaaccaccctcggtgcgatttccccatccactggccgtaccctgccagaccgctacattgaaggcacctgcccaatctgtggcaccgacggcgctcgtggcgaccagtgcgacaactgcggaaaccagctcgatccagcggacctgatcaacccggtgtccaagatcaacggcgaaaccccagagttcgttgagaccgaacacttcctgctcgacctgccagcactagctgaagcactaaccgagtggctgaagggacgcgaagactggcgtccaaacgtgttgaagttctcgctcaacctgctggacgatatccgcccacgcgcaatgtcgcgcgatat